European Patent Specification EP 3 313 420 B1, published March 13, 2024. Title: METHODS AND COMPOSITIONS RELATING TO HEMATOPOIETIC STEM CELL EXPANSION, ENRICHMENT, AND MAINTENANCE. Applicant: CHILDREN'S MEDICAL CENTER CORPORATION. The sequence listing filed with the application follows.

SEQUENCE LISTING (13 sequences)

SEQ ID NO: 1 - DNA, 21 bp, Homo sapiens
aatcctgcatgagcaactgca

SEQ ID NO: 2 - DNA, 21 bp, Artificial Sequence
  Description of Artificial Sequence: Synthetic oligonucleotide
  Description of Combined DNA/RNA Molecule: Synthetic oligonucleotide
uccugcaugagcaacugcatt

SEQ ID NO: 3 - DNA, 21 bp, Artificial Sequence
  Description of Artificial Sequence: Synthetic oligonucleotide
  Description of Combined DNA/RNA Molecule: Synthetic oligonucleotide
ugcaguugcucaugcaggatt

SEQ ID NO: 4 - DNA, 21 bp, Homo sapiens
aaggccaagctgaagcagaac

SEQ ID NO: 5 - DNA, 21 bp, Artificial Sequence
  Description of Artificial Sequence: Synthetic oligonucleotide
  Description of Combined DNA/RNA Molecule: Synthetic oligonucleotide
ggccaagcugaagcagaactt

SEQ ID NO: 6 - DNA, 21 bp, Artificial Sequence
  Description of Artificial Sequence: Synthetic oligonucleotide
  Description of Combined DNA/RNA Molecule: Synthetic oligonucleotide
guucugcuucagcuuggcctt

SEQ ID NO: 7 - DNA, 20 bp, Homo sapiens
agcatgagaacatactccag

SEQ ID NO: 8 - DNA, 21 bp, Artificial Sequence
  Description of Artificial Sequence: Synthetic oligonucleotide
  Description of Combined DNA/RNA Molecule: Synthetic oligonucleotide
gcaugagaacauacuccagtt

SEQ ID NO: 9 - DNA, 21 bp, Artificial Sequence
  Description of Artificial Sequence: Synthetic oligonucleotide
  Description of Combined DNA/RNA Molecule: Synthetic oligonucleotide
cuggaguauguucucaugctt

SEQ ID NO: 10 - DNA, 21 bp, Homo sapiens
aagacgcggaagctcatggag

SEQ ID NO: 11 - DNA, 21 bp, Artificial Sequence
  Description of Artificial Sequence: Synthetic oligonucleotide
  Description of Combined DNA/RNA Molecule: Synthetic oligonucleotide
gacgcggaagcucauggagtt

SEQ ID NO: 12 - DNA, 21 bp, Artificial Sequence
  Description of Artificial Sequence: Synthetic oligonucleotide
  Description of Combined DNA/RNA Molecule: Synthetic oligonucleotide
cuccaugagcuuccgcguctt

SEQ ID NO: 13 - protein, 14 aa, Artificial Sequence
  Description of Artificial Sequence: Synthetic peptide
  N-term Ac
  MISC_FEATURE (3)..(10): Cross-link between residues
  C-term NH2
PQRILDQHVSRVMK